European Patent Specification EP 4 281 588 B1, published May 21, 2025. Title: A method for diagnosing endometrial or ovarian carcinoma. Applicant: Université de Paris et al. The sequence listing filed with the application follows.

SEQUENCE LISTING (11 sequences)

SEQ ID NO: 1 - DNA, 90 bp, Artificial Sequence
  probe cg06404175 on position chr20:3072046
ttttcgagcgagtttttagcgtcgtttcggttttcgtttatttcgttcgttttcgtagtgttttttttgcggtttcgggggtaaaggtcg

SEQ ID NO: 2 - DNA, 87 bp, Artificial Sequence
  probe cg25060829 on position chr6:28399794
ataaaggtcggaagcggttacggggggtttaagaattagttcgcgcggggcgtattttcgcggtcgttttaggaagggagcgaaagg

SEQ ID NO: 3 - DNA, 20 bp, Artificial Sequence
  probe sequence for ZSCAN12
ttaagaattagttcgcgcgg

SEQ ID NO: 4 - DNA, 23 bp, Artificial Sequence
  probe sequence for OXT
tcggttttcgtttatttcgttcg

SEQ ID NO: 5 - DNA, 17 bp, Artificial Sequence
  probe sequence for ALB
agggtttttataattta

SEQ ID NO: 6 - DNA, 20 bp, Artificial Sequence
  forward primer sequence for ZSCAN12
ataaaggtcggaagcggtta

SEQ ID NO: 7 - DNA, 20 bp, Artificial Sequence
  reverse primer sequence for ZSCAN12
cctttcgctcccttcctaaa

SEQ ID NO: 8 - DNA, 21 bp, Artificial Sequence
  forward primer sequence for OXT
ttttcgagcgagtttttagcg

SEQ ID NO: 9 - DNA, 19 bp, Artificial Sequence
  reverse primer sequence for OXT
cgacctttacccccgaaac

SEQ ID NO: 10 - DNA, 22 bp, Artificial Sequence
  forward primer sequence for ALB
gggatggaaagaattttatgtt

SEQ ID NO: 11 - DNA, 22 bp, Artificial Sequence
  reverse primer sequence for ALB
aaacaaactaaccccaaattct